European Patent Application EP 4 163 635 A1, published April 12, 2023. Title: Sensing platform. Applicant: ECOLE POLYTECHNIQUE FEDERALE DE LAUSANNE. The sequence listing filed with the application follows.

SEQUENCE LISTING (19 sequences)

SEQ ID NO: 1 - protein, 583 aa, Aspergillus niger
SNGIEASLLTDPKDVSGRTVDYIIAGGGLTGLTTAARLTENPNISVLVIESGSYESDRGPIIEDLNAYGDIFGSSVDHAYETVELATNNQTALIRSGNGLGGSTLVNGGTWTRPHKAQVDSWETVFGNEGWNWDNVAAYSLQAERARAPNAKQIAAGHYFNASCHGVNGTVHAGPRDTGDDYSPIVKALMSAVEDRGVPTKKDFGCGDPHGVSMFPNTLHEDQVRSDAAREWLLPNYQRPNLQVLTGQYVGKVLLSQNGTTPRAVGVEFGTHKGNTHNVYAKHEVLLAAGSAVSPTILEYSGIGMKSILEPLGIDTVVDLPVGLNLQDQTTATVRSRITSAGAGQGQAAWFATFNETFGDYSEKAHELLNTKLEQWAEEAVARGGFHNTTALLIQYENYRDWIVNHNVAYSELFLDTAGVASFDVWDLLPFTRGYVHILDKDPYLHHFAYDPQYFLNELDLLGQAAATQLARNISNSGAMQTYFAGETIPGDNLAYDADLSAWTEYIPYHFRPNYHGVGTCSMMPKEMGGVVDNAARVYGVQGLRVIDGSIPPTQMSSHVMTVFYAMALKISDAILEDYASMQ

SEQ ID NO: 2 - protein, 583 aa, Aspergillus niger
  misc (13)..(13): X is selected from a cysteine or an amino acid including a thiol or selenol group, for example selenocysteine
  misc (13)..(13): X is selected from a cysteine or an amino acid including a thiol or selenol group, for example selenocysteine
SNGIEASLLTDPXDVSGRTVDYIIAGGGLTGLTTAARLTENPNISVLVIESGSYESDRGPIIEDLNAYGDIFGSSVDHAYETVELATNNQTALIRSGNGLGGSTLVNGGTWTRPHKAQVDSWETVFGNEGWNWDNVAAYSLQAERARAPNAKQIAAGHYFNASCHGVNGTVHAGPRDTGDDYSPIVKALMSAVEDRGVPTKKDFGCGDPHGVSMFPNTLHEDQVRSDAAREWLLPNYQRPNLQVLTGQYVGKVLLSQNGTTPRAVGVEFGTHKGNTHNVYAKHEVLLAAGSAVSPTILEYSGIGMKSILEPLGIDTVVDLPVGLNLQDQTTATVRSRITSAGAGQGQAAWFATFNETFGDYSEKAHELLNTKLEQWAEEAVARGGFHNTTALLIQYENYRDWIVNHNVAYSELFLDTAGVASFDVWDLLPFTRGYVHILDKDPYLHHFAYDPQYFLNELDLLGQAAATQLARNISNSGAMQTYFAGETIPGDNLAYDADLSAWTEYIPYHFRPNYHGVGTCSMMPKEMGGVVDNAARVYGVQGLRVIDGSIPPTQMSSHVMTVFYAMALKISDAILEDYASMQ

SEQ ID NO: 3 - protein, 583 aa, Aspergillus niger
  misc (70)..(70): X is selected from a cysteine or an amino acid including a thiol or selenol group, for example selenocysteine
SNGIEASLLTDPKDVSGRTVDYIIAGGGLTGLTTAARLTENPNISVLVIESGSYESDRGPIIEDLNAYGXIFGSSVDHAYETVELATNNQTALIRSGNGLGGSTLVNGGTWTRPHKAQVDSWETVFGNEGWNWDNVAAYSLQAERARAPNAKQIAAGHYFNASCHGVNGTVHAGPRDTGDDYSPIVKALMSAVEDRGVPTKKDFGCGDPHGVSMFPNTLHEDQVRSDAAREWLLPNYQRPNLQVLTGQYVGKVLLSQNGTTPRAVGVEFGTHKGNTHNVYAKHEVLLAAGSAVSPTILEYSGIGMKSILEPLGIDTVVDLPVGLNLQDQTTATVRSRITSAGAGQGQAAWFATFNETFGDYSEKAHELLNTKLEQWAEEAVARGGFHNTTALLIQYENYRDWIVNHNVAYSELFLDTAGVASFDVWDLLPFTRGYVHILDKDPYLHHFAYDPQYFLNELDLLGQAAATQLARNISNSGAMQTYFAGETIPGDNLAYDADLSAWTEYIPYHFRPNYHGVGTCSMMPKEMGGVVDNAARVYGVQGLRVIDGSIPPTQMSSHVMTVFYAMALKISDAILEDYASMQ

SEQ ID NO: 4 - protein, 583 aa, Aspergillus niger
  misc (418)..(418): X is selected from a cysteine or an amino acid including a thiol or selenol group, for example selenocysteine
SNGIEASLLTDPKDVSGRTVDYIIAGGGLTGLTTAARLTENPNISVLVIESGSYESDRGPIIEDLNAYGDIFGSSVDHAYETVELATNNQTALIRSGNGLGGSTLVNGGTWTRPHKAQVDSWETVFGNEGWNWDNVAAYSLQAERARAPNAKQIAAGHYFNASCHGVNGTVHAGPRDTGDDYSPIVKALMSAVEDRGVPTKKDFGCGDPHGVSMFPNTLHEDQVRSDAAREWLLPNYQRPNLQVLTGQYVGKVLLSQNGTTPRAVGVEFGTHKGNTHNVYAKHEVLLAAGSAVSPTILEYSGIGMKSILEPLGIDTVVDLPVGLNLQDQTTATVRSRITSAGAGQGQAAWFATFNETFGDYSEKAHELLNTKLEQWAEEAVARGGFHNTTALLIQYENYRDWIVNHNVAYSELFLDTXGVASFDVWDLLPFTRGYVHILDKDPYLHHFAYDPQYFLNELDLLGQAAATQLARNISNSGAMQTYFAGETIPGDNLAYDADLSAWTEYIPYHFRPNYHGVGTCSMMPKEMGGVVDNAARVYGVQGLRVIDGSIPPTQMSSHVMTVFYAMALKISDAILEDYASMQ

SEQ ID NO: 5 - protein, 583 aa, Aspergillus niger
  misc (446)..(446): X is selected from a cysteine or an amino acid including a thiol or selenol group, for example selenocysteine
SNGIEASLLTDPKDVSGRTVDYIIAGGGLTGLTTAARLTENPNISVLVIESGSYESDRGPIIEDLNAYGDIFGSSVDHAYETVELATNNQTALIRSGNGLGGSTLVNGGTWTRPHKAQVDSWETVFGNEGWNWDNVAAYSLQAERARAPNAKQIAAGHYFNASCHGVNGTVHAGPRDTGDDYSPIVKALMSAVEDRGVPTKKDFGCGDPHGVSMFPNTLHEDQVRSDAAREWLLPNYQRPNLQVLTGQYVGKVLLSQNGTTPRAVGVEFGTHKGNTHNVYAKHEVLLAAGSAVSPTILEYSGIGMKSILEPLGIDTVVDLPVGLNLQDQTTATVRSRITSAGAGQGQAAWFATFNETFGDYSEKAHELLNTKLEQWAEEAVARGGFHNTTALLIQYENYRDWIVNHNVAYSELFLDTAGVASFDVWDLLPFTRGYVHILDKDPYLXHFAYDPQYFLNELDLLGQAAATQLARNISNSGAMQTYFAGETIPGDNLAYDADLSAWTEYIPYHFRPNYHGVGTCSMMPKEMGGVVDNAARVYGVQGLRVIDGSIPPTQMSSHVMTVFYAMALKISDAILEDYASMQ

SEQ ID NO: 6 - protein, 605 aa, Aspergillus niger
MQTLLVSSLVVSLAAALPHYIRSNGIEASLLTDPKDVSGRTVDYIIAGGGLTGLTTAARLTENPNISVLVIESGSYESDRGPIIEDLNAYGDIFGSSVDHAYETVELATNNQTALIRSGNGLGGSTLVNGGTWTRPHKAQVDSWETVFGNEGWNWDNVAAYSLQAERARAPNAKQIAAGHYFNASCHGVNGTVHAGPRDTGDDYSPIVKALMSAVEDRGVPTKKDFGCGDPHGVSMFPNTLHEDQVRSDAAREWLLPNYQRPNLQVLTGQYVGKVLLSQNGTTPRAVGVEFGTHKGNTHNVYAKHEVLLAAGSAVSPTILEYSGIGMKSILEPLGIDTVVDLPVGLNLQDQTTATVRSRITSAGAGQGQAAWFATFNETFGDYSEKAHELLNTKLEQWAEEAVARGGFHNTTALLIQYENYRDWIVNHNVAYSELFLDTAGVASFDVWDLLPFTRGYVHILDKDPYLHHFAYDPQYFLNELDLLGQAAATQLARNISNSGAMQTYFAGETIPGDNLAYDADLSAWTEYIPYHFRPNYHGVGTCSMMPKEMGGVVDNAARVYGVQGLRVIDGSIPPTQMSSHVMTVFYAMALKISDAILEDYASMQ

SEQ ID NO: 7 - DNA, 1752 bp, Aspergillus niger
tctaatggtattgaggcatctcttttgactgaccctaaggacgtctcaggtcgtaccgttgattatatcattgctggaggtggtttgaccggtcttactactgcagctagactgaccgaaaacccaaacatctccgtgttggttatcgaatccggttcctatgaatctgacagaggtccaatcattgaggacttgaatgcttatggtgacatcttcggatcttctgttgaccacgcttatgaaactgtcgagttagctactaacaaccaaactgcattgatcagatctggaaatggtttgggtggttccacccttgttaacggtggaacctggacccgtcctcacaaggctcaggtcgattcctgggaaactgttttcggtaacgaaggatggaattgggacaatgttgctgcttactctcttcaagctgagagagcacgtgctccaaacgccaagcaaatcgctgctggacactacttcaacgcctcatgccacggtgtcaatggaactgtgcacgctggtcctagagataccggagacgactattctcctattgttaaggctctgatgtctgctgttgaagacagaggtgttcctaccaagaaagacttcggttgcggtgatcctcacggtgtgtccatgtttcctaacaccttgcatgaggaccaggtgagatccgatgcagctagagagtggcttcttcctaactaccaacgtcctaacttgcaggtcttgactggtcagtacgttggaaaggttcttttgtcccagaatggtactacccctcgtgctgtgggtgttgagttcggtactcacaagggtaacactcacaacgtttacgccaagcacgaggtgcttttggcagctggttccgcagtttcccctactattctggagtactcaggtattggtatgaagtctattcttgaaccattgggtattgatactgtcgttgacttgccagttggtttgaacttgcaagaccaaaccactgctactgttagatccagaatcacttctgctggtgctggtcaaggtcaagctgcttggtttgccactttcaacgaaactttcggtgactattccgaaaaggctcacgaattgttgaacaccaaactggaacagtgggctgaagaggctgtcgctagaggtggttttcacaacaccaccgctttgttgatccagtacgaaaactacagagactggatcgttaaccacaacgttgcctactctgaattgttccttgacactgcaggtgtcgcttcttttgacgtgtgggacttgttgcctttcaccagaggttacgttcacatcttggacaaggacccataccttcaccacttcgcttacgaccctcaatacttccttaacgagctggacttgcttggacaagctgctgctactcaattggcaagaaacatctctaactccggagccatgcagacctacttcgctggagaaactatccctggtgacaacttagcttacgatgctgacctttctgcatggaccgaatacattccataccacttccgtccaaactaccacggagtgggtacctgttctatgatgccaaaggaaatgggtggagttgttgacaatgctgctcgtgtctatggtgttcaaggtcttagagttatcgatggttccatccctcctactcaaatgtcttcacatgtgatgaccgtcttctacgctatggccttgaagatttctgacgcaatcttggaggactacgcatctatgcaataa

SEQ ID NO: 8 - DNA, 1752 bp, Aspergillus niger
tctaatggtattgaggcatctcttttgactgacccttgtgacgtctcaggtcgtaccgttgattatatcattgctggaggtggtttgaccggtcttactactgcagctagactgaccgaaaacccaaacatctccgtgttggttatcgaatccggttcctatgaatctgacagaggtccaatcattgaggacttgaatgcttatggtgacatcttcggatcttctgttgaccacgcttatgaaactgtcgagttagctactaacaaccaaactgcattgatcagatctggaaatggtttgggtggttccacccttgttaacggtggaacctggacccgtcctcacaaggctcaggtcgattcctgggaaactgttttcggtaacgaaggatggaattgggacaatgttgctgcttactctcttcaagctgagagagcacgtgctccaaacgccaagcaaatcgctgctggacactacttcaacgcctcatgccacggtgtcaatggaactgtgcacgctggtcctagagataccggagacgactattctcctattgttaaggctctgatgtctgctgttgaagacagaggtgttcctaccaagaaagacttcggttgcggtgatcctcacggtgtgtccatgtttcctaacaccttgcatgaggaccaggtgagatccgatgcagctagagagtggcttcttcctaactaccaacgtcctaacttgcaggtcttgactggtcagtacgttggaaaggttcttttgtcccagaatggtactacccctcgtgctgtgggtgttgagttcggtactcacaagggtaacactcacaacgtttacgccaagcacgaggtgcttttggcagctggttccgcagtttcccctactattctggagtactcaggtattggtatgaagtctattcttgaaccattgggtattgatactgtcgttgacttgccagttggtttgaacttgcaagaccaaaccactgctactgttagatccagaatcacttctgctggtgctggtcaaggtcaagctgcttggtttgccactttcaacgaaactttcggtgactattccgaaaaggctcacgaattgttgaacaccaaactggaacagtgggctgaagaggctgtcgctagaggtggttttcacaacaccaccgctttgttgatccagtacgaaaactacagagactggatcgttaaccacaacgttgcctactctgaattgttccttgacactgcaggtgtcgcttcttttgacgtgtgggacttgttgcctttcaccagaggttacgttcacatcttggacaaggacccataccttcaccacttcgcttacgaccctcaatacttccttaacgagctggacttgcttggacaagctgctgctactcaattggcaagaaacatctctaactccggagccatgcagacctacttcgctggagaaactatccctggtgacaacttagcttacgatgctgacctttctgcatggaccgaatacattccataccacttccgtccaaactaccacggagtgggtacctgttctatgatgccaaaggaaatgggtggagttgttgacaatgctgctcgtgtctatggtgttcaaggtcttagagttatcgatggttccatccctcctactcaaatgtcttcacatgtgatgaccgtcttctacgctatggccttgaagatttctgacgcaatcttggaggactacgcatctatgcaataa

SEQ ID NO: 9 - DNA, 1752 bp, Aspergillus niger
tctaatggtattgaggcatctcttttgactgaccctaaggacgtctcaggtcgtaccgttgattatatcattgctggaggtggtttgaccggtcttactactgcagctagactgaccgaaaacccaaacatctccgtgttggttatcgaatccggttcctatgaatctgacagaggtccaatcattgaggacttgaatgcttatggttgtatcttcggatcttctgttgaccacgcttatgaaactgtcgagttagctactaacaaccaaactgcattgatcagatctggaaatggtttgggtggttccacccttgttaacggtggaacctggacccgtcctcacaaggctcaggtcgattcctgggaaactgttttcggtaacgaaggatggaattgggacaatgttgctgcttactctcttcaagctgagagagcacgtgctccaaacgccaagcaaatcgctgctggacactacttcaacgcctcatgccacggtgtcaatggaactgtgcacgctggtcctagagataccggagacgactattctcctattgttaaggctctgatgtctgctgttgaagacagaggtgttcctaccaagaaagacttcggttgcggtgatcctcacggtgtgtccatgtttcctaacaccttgcatgaggaccaggtgagatccgatgcagctagagagtggcttcttcctaactaccaacgtcctaacttgcaggtcttgactggtcagtacgttggaaaggttcttttgtcccagaatggtactacccctcgtgctgtgggtgttgagttcggtactcacaagggtaacactcacaacgtttacgccaagcacgaggtgcttttggcagctggttccgcagtttcccctactattctggagtactcaggtattggtatgaagtctattcttgaaccattgggtattgatactgtcgttgacttgccagttggtttgaacttgcaagaccaaaccactgctactgttagatccagaatcacttctgctggtgctggtcaaggtcaagctgcttggtttgccactttcaacgaaactttcggtgactattccgaaaaggctcacgaattgttgaacaccaaactggaacagtgggctgaagaggctgtcgctagaggtggttttcacaacaccaccgctttgttgatccagtacgaaaactacagagactggatcgttaaccacaacgttgcctactctgaattgttccttgacactgcaggtgtcgcttcttttgacgtgtgggacttgttgcctttcaccagaggttacgttcacatcttggacaaggacccataccttcaccacttcgcttacgaccctcaatacttccttaacgagctggacttgcttggacaagctgctgctactcaattggcaagaaacatctctaactccggagccatgcagacctacttcgctggagaaactatccctggtgacaacttagcttacgatgctgacctttctgcatggaccgaatacattccataccacttccgtccaaactaccacggagtgggtacctgttctatgatgccaaaggaaatgggtggagttgttgacaatgctgctcgtgtctatggtgttcaaggtcttagagttatcgatggttccatccctcctactcaaatgtcttcacatgtgatgaccgtcttctacgctatggccttgaagatttctgacgcaatcttggaggactacgcatctatgcaataa

SEQ ID NO: 10 - DNA, 1752 bp, Aspergillus niger
tctaatggtattgaggcatctcttttgactgaccctaaggacgtctcaggtcgtaccgttgattatatcattgctggaggtggtttgaccggtcttactactgcagctagactgaccgaaaacccaaacatctccgtgttggttatcgaatccggttcctatgaatctgacagaggtccaatcattgaggacttgaatgcttatggtgacatcttcggatcttctgttgaccacgcttatgaaactgtcgagttagctactaacaaccaaactgcattgatcagatctggaaatggtttgggtggttccacccttgttaacggtggaacctggacccgtcctcacaaggctcaggtcgattcctgggaaactgttttcggtaacgaaggatggaattgggacaatgttgctgcttactctcttcaagctgagagagcacgtgctccaaacgccaagcaaatcgctgctggacactacttcaacgcctcatgccacggtgtcaatggaactgtgcacgctggtcctagagataccggagacgactattctcctattgttaaggctctgatgtctgctgttgaagacagaggtgttcctaccaagaaagacttcggttgcggtgatcctcacggtgtgtccatgtttcctaacaccttgcatgaggaccaggtgagatccgatgcagctagagagtggcttcttcctaactaccaacgtcctaacttgcaggtcttgactggtcagtacgttggaaaggttcttttgtcccagaatggtactacccctcgtgctgtgggtgttgagttcggtactcacaagggtaacactcacaacgtttacgccaagcacgaggtgcttttggcagctggttccgcagtttcccctactattctggagtactcaggtattggtatgaagtctattcttgaaccattgggtattgatactgtcgttgacttgccagttggtttgaacttgcaagaccaaaccactgctactgttagatccagaatcacttctgctggtgctggtcaaggtcaagctgcttggtttgccactttcaacgaaactttcggtgactattccgaaaaggctcacgaattgttgaacaccaaactggaacagtgggctgaagaggctgtcgctagaggtggttttcacaacaccaccgctttgttgatccagtacgaaaactacagagactggatcgttaaccacaacgttgcctactctgaattgttccttgacacttgtggtgtcgcttcttttgacgtgtgggacttgttgcctttcaccagaggttacgttcacatcttggacaaggacccataccttcaccacttcgcttacgaccctcaatacttccttaacgagctggacttgcttggacaagctgctgctactcaattggcaagaaacatctctaactccggagccatgcagacctacttcgctggagaaactatccctggtgacaacttagcttacgatgctgacctttctgcatggaccgaatacattccataccacttccgtccaaactaccacggagtgggtacctgttctatgatgccaaaggaaatgggtggagttgttgacaatgctgctcgtgtctatggtgttcaaggtcttagagttatcgatggttccatccctcctactcaaatgtcttcacatgtgatgaccgtcttctacgctatggccttgaagatttctgacgcaatcttggaggactacgcatctatgcaataa

SEQ ID NO: 11 - DNA, 1752 bp, Aspergillus niger
tctaatggtattgaggcatctcttttgactgaccctaaggacgtctcaggtcgtaccgttgattatatcattgctggaggtggtttgaccggtcttactactgcagctagactgaccgaaaacccaaacatctccgtgttggttatcgaatccggttcctatgaatctgacagaggtccaatcattgaggacttgaatgcttatggtgacatcttcggatcttctgttgaccacgcttatgaaactgtcgagttagctactaacaaccaaactgcattgatcagatctggaaatggtttgggtggttccacccttgttaacggtggaacctggacccgtcctcacaaggctcaggtcgattcctgggaaactgttttcggtaacgaaggatggaattgggacaatgttgctgcttactctcttcaagctgagagagcacgtgctccaaacgccaagcaaatcgctgctggacactacttcaacgcctcatgccacggtgtcaatggaactgtgcacgctggtcctagagataccggagacgactattctcctattgttaaggctctgatgtctgctgttgaagacagaggtgttcctaccaagaaagacttcggttgcggtgatcctcacggtgtgtccatgtttcctaacaccttgcatgaggaccaggtgagatccgatgcagctagagagtggcttcttcctaactaccaacgtcctaacttgcaggtcttgactggtcagtacgttggaaaggttcttttgtcccagaatggtactacccctcgtgctgtgggtgttgagttcggtactcacaagggtaacactcacaacgtttacgccaagcacgaggtgcttttggcagctggttccgcagtttcccctactattctggagtactcaggtattggtatgaagtctattcttgaaccattgggtattgatactgtcgttgacttgccagttggtttgaacttgcaagaccaaaccactgctactgttagatccagaatcacttctgctggtgctggtcaaggtcaagctgcttggtttgccactttcaacgaaactttcggtgactattccgaaaaggctcacgaattgttgaacaccaaactggaacagtgggctgaagaggctgtcgctagaggtggttttcacaacaccaccgctttgttgatccagtacgaaaactacagagactggatcgttaaccacaacgttgcctactctgaattgttccttgacactgcaggtgtcgcttcttttgacgtgtgggacttgttgcctttcaccagaggttacgttcacatcttggacaaggacccatacctttgtcacttcgcttacgaccctcaatacttccttaacgagctggacttgcttggacaagctgctgctactcaattggcaagaaacatctctaactccggagccatgcagacctacttcgctggagaaactatccctggtgacaacttagcttacgatgctgacctttctgcatggaccgaatacattccataccacttccgtccaaactaccacggagtgggtacctgttctatgatgccaaaggaaatgggtggagttgttgacaatgctgctcgtgtctatggtgttcaaggtcttagagttatcgatggttccatccctcctactcaaatgtcttcacatgtgatgaccgtcttctacgctatggccttgaagatttctgacgcaatcttggaggactacgcatctatgcaataa

SEQ ID NO: 12 - DNA, 27 bp, Artificial Sequence
  K13C-F  primer sequence
ggactgacccttgtgacgtctcaggtc

SEQ ID NO: 13 - DNA, 27 bp, Artificial Sequence
  K13C-R  primer sequence
gacctgagacgtcacaagggtcagtcc

SEQ ID NO: 14 - DNA, 30 bp, Artificial Sequence
  D70C-F  primer sequence
gaatgcttatggttgtatcttcggatcttc

SEQ ID NO: 15 - DNA, 30 bp, Artificial Sequence
  D70C-R  primer sequence
gaagatccgaagatacaaccataagcattc

SEQ ID NO: 16 - DNA, 27 bp, Artificial Sequence
  A418C-F  primer sequence
gacctgagacgtcacaagggtcagtcc

SEQ ID NO: 17 - DNA, 27 bp, Artificial Sequence
  A418C-R primer sequence
gttccttgacacttgtggtgtcgcttc

SEQ ID NO: 18 - DNA, 29 bp, Artificial Sequence
  H446C-F primer sequence
ggacccatacctttgtcacttcgcttacg

SEQ ID NO: 19 - DNA, 29 bp, Artificial Sequence
  H446C-R  primer sequence
cgtaagcgaagtgacaaaggtatgggtcc